European Patent Application EP 4 703 466 A1, published March 4, 2026. Title: 靶向CLL1的CAR-T细胞及其制备方法与应用. Applicant: 浙江康佰裕生物科技有限公司. Application CN. The sequence listing filed with the application follows.

SEQUENCE LISTING (2 sequences)

SEQ ID NO: 1 - protein, 378 aa, synthetic construct
MALPVTALLLPLALLLHAARPDVQLQESGGGLVQPGGSLRLSCAASGFTFGSYDMTWVRQAPGKGPEWVSGINSGGSSTYYADSVKGRFTISRDNAKNTLYLQMNSLKPEDTAVYYCATIDRLSTVVAGTYQPSEEYDYWGQGTQVTVSSTTTPAPRPPTPAPTIASQPLSLRPEACRPAAGGAVHTRGLDFACDIYIWAPLAGTCGVLLLSLVITLYCRFSVVKRGRKKLLYIFKQPFMRPVQTTQEEDGCSCRFPEEEEGGCELRVKFSRSADAPAYQQGQNQLYNELNLGRREEYDVLDKRRGRDPEMGGKPRRKNPQEGLYNELQKDKMAEAYSEIGMKGERRRGKGHDGLYQGLSTATKDTYDALHMQALPPR

SEQ ID NO: 2 - DNA, 1134 bp, synthetic construct
  source 1..1134: mol_type = other DNA
atggctctgcctgtgaccgccctgctgctgcctctggctctgctgctgcacgccgctcggcctgatgtgcagctgcaggagtctggaggaggcttggtgcagcctgggggttctctgagactctcctgtgcagcctctggattcaccttcggaagctatgacatgacctgggtccgccaggctccaggaaaggggcccgagtgggtctcaggaattaatagtggtggtagtagcacatactatgcagactccgtgaagggccgattcaccatctccagagacaacgccaagaacacgctgtatctgcaaatgaacagcctgaaacctgaggacacggccgtgtattactgtgcaactatcgaccgccttagtacggtagtagctggtacgtaccagccgtccgaagaatatgactactggggccaggggacccaggtcaccgtctccagcactacaactccagcacccagaccccctacacctgctccaactatcgcaagtcagcccctgtcactgcgccctgaagcctgtcgccctgctgccgggggagctgtgcatactcggggactggactttgcctgtgatatctacatctgggcgcccttggccgggacttgtggggtccttctcctgtcactggttatcaccctttactgcaggttcagtgtcgtgaagagaggccggaagaagctgctgtacatcttcaagcagcctttcatgaggcccgtgcagactacccaggaggaagatggatgcagctgtagattccctgaagaggaggaaggaggctgtgagctgagagtgaagttctcccgaagcgcagatgccccagcctatcagcagggacagaatcagctgtacaacgagctgaacctgggaagacgggaggaatacgatgtgctggacaaaaggcggggcagagatcctgagatgggcggcaaaccaagacggaagaacccccaggaaggtctgtataatgagctgcagaaagacaagatggctgaggcctactcagaaatcgggatgaagggcgaaagaaggagaggaaaaggccacgacggactgtaccaggggctgagtacagcaacaaaagacacctatgacgctctgcacatgcaggctctgccaccaaga